European Patent Application EP 4 599 885 A2, published August 13, 2025. Title: Compounds for the treatment of glioblastoma. Applicant: Merck Patent GmbH. Application EP EP25168445.2, filed April 4, 2025. The sequence listing filed with the application follows.

SEQUENCE LISTING (8 sequences)

SEQ ID NO: 1 - DNA, 22 bp, synthetic construct
  source 1..22: mol_type = other DNA
cctaagatgagcgcaagttgaa

SEQ ID NO: 2 - DNA, 24 bp, synthetic construct
  source 1..24: mol_type = other DNA
ccacaggactagaacacctgctaa

SEQ ID NO: 3 - DNA, 24 bp, synthetic construct
  source 1..24: mol_type = other DNA
tcaaaatgtcacctaaaacaatcc

SEQ ID NO: 4 - DNA, 24 bp, synthetic construct
  source 1..24: mol_type = other DNA
acaaacaatacaacagaaaacacc

SEQ ID NO: 5 - DNA, 21 bp, synthetic construct
  source 1..21: mol_type = other DNA
tttggggaagtctcatttttg

SEQ ID NO: 6 - DNA, 20 bp, synthetic construct
  source 1..20: mol_type = other DNA
cgattttcagttggcttttg

SEQ ID NO: 7 - RNA, 20 nt, synthetic construct
  source 1..20: mol_type = other RNA
cgattttcagttggcttttg

SEQ ID NO: 8 - RNA, 20 nt, synthetic construct
  source 1..20: mol_type = other RNA
gtatcggacagagtttacca